European Patent Application EP 4 434 546 A1, published September 25, 2024. Title: 新型酸敏感性适配体雷公藤甲素偶联物及应用. Applicant: 成都中医药大学. The sequence listing filed with the application follows.

SEQUENCE LISTING (9 sequences)

SEQ ID NO: 1 - DNA, 26 bp, synthetic construct
  source 1..26: mol_type = other DNA
ggtggtggtggttgtggtggtggtgg

SEQ ID NO: 2 - RNA, 29 nt, synthetic construct
  source 1..29: mol_type = other RNA
gcgaaccgatggaatttttggacgctcgc

SEQ ID NO: 3 - DNA, 41 bp, synthetic construct
  source 1..41: mol_type = other DNA
atctaactgctgcgccgccgggaaaatactgtacggttaga

SEQ ID NO: 4 - RNA, 71 nt, synthetic construct
  source 1..71: mol_type = other RNA
gggaggacgatgcggatcagccatgtttacgtcactccttgtcaatcctcatcggcagacgactcgcccga

SEQ ID NO: 5 - DNA, 72 bp, synthetic construct
  source 1..72: mol_type = other DNA
gggagacaagaataaacgctcaannnnnnnnnnnnnnnnnnnnnnnnnttcgacaggaggctcacaacaggc

SEQ ID NO: 6 - RNA, 34 nt, synthetic construct
  source 1..34: mol_type = other RNA
gggggcatacttgtgagacttttatgtcaccccc

SEQ ID NO: 7 - RNA, 39 nt, synthetic construct
  source 1..39: mol_type = other RNA
gccttagtaacgtgctttgatgtcgattcgacaggaggc

SEQ ID NO: 8 - DNA, 25 bp, synthetic construct
  source 1..25: mol_type = other DNA
gcagttgatcctttggataccctgg

SEQ ID NO: 9 - RNA, 48 nt, synthetic construct
  source 1..48: mol_type = other RNA
ggacggatttaatcgccgtagaaaagcatgtcaaagccggaaccgtcc